European Patent Application EP 4 242 302 A1, published September 13, 2023. Title: Modified polypeptide having mannanase activity. Applicant: CJ CheilJedang Corporation. The sequence listing filed with the application follows.

SEQUENCE LISTING (16 sequences)

SEQ ID NO: 1 - protein, 345 aa, synthetic construct
  REGION 1..345: note = Mannanase
SFASTSGLQFTIDGETGYFAGTNSYWIGFLTDNADVDLVMGHLKSSGLKILRVWGFNDVTSQPSSGTVWYQLHQDGKSTINTGADGLQRLDYVVSSAEQHDIKLIINFVNYWTDYGGMSAYVSAYGGSGETDFYTSDTMQSAYQTYIKTVVERYSNSSAVFAWELANEPRCPSCDTSVLYNWIEKTSKFIKGLDADRMVCIGDEGFGLNIDSDGSYPYQFSEGLNFTMNLGIDTIDFGTLHLYPDSWGTSDDWGNGWITAHGAACKAAGKPCLLEEYGVTSNHCSVEGSWQKTALSTTGVGADLFWQYGDDLSTGKSPDDGNTIYYGTSDYQCLVTDHVAAIGSA

SEQ ID NO: 2 - DNA, 1035 bp, synthetic construct
  misc_feature 1..1035: note = Mannanase
  source 1..1035: mol_type = other DNA
agttttgcttctacatcaggactacaattcaccatcgatggtgagacaggttatttcgccggtacaaatagttactggatcggttttctgaccgacaacgcagatgtggatcttgttatgggtcatctgaaaagcagcggcttgaagatcctgcgtgtatggggtttcaacgacgttacctctcagccgagcagcgggacggtctggtatcaactgcaccaagatggaaaaagcaccattaacaccggtgcggatggcctccagcgtctggattacgtcgtgagcagcgctgaacagcacgatatcaaactgattattaacttcgtgaactattggaccgactacggcggtatgagcgcgtacgtgagcgcgtacggcggctctggcgaaaccgatttctacacctcggataccatgcagagcgcgtaccaaacctatatcaaaaccgtggtggagcgctatagcaacagcagcgctgtgtttgcttgggaactggcaaatgaaccgcgttgcccgtcttgtgatacctccgtgctgtacaactggatcgagaaaacctccaaattcatcaagggtttagacgccgaccgcatggtttgcattggcgatgagggtttcggcctgaacatcgacagcgatggcagctacccgtatcagtttagcgaaggcctgaattttaccatgaatctgggtattgacaccatcgattttggtacgttgcatctgtacccagattcctggggtacgtccgacgactggggcaacggttggattaccgcacatggtgctgcgtgtaaagcagccggtaagccgtgcctgctggaagagtatggtgttaccagcaatcattgcagcgttgagggcagttggcaaaaaactgcgctgagcacgaccggtgttggtgcggatctgttttggcagtatggcgatgacctctcaacgggcaaatccccggatgatggcaacactatttattacggcacctctgactaccaatgtctggttactgaccacgtcgcggcgattggttctgcg

SEQ ID NO: 3 - protein, 345 aa, synthetic construct
  REGION 1..345: note = Mannanase variant
SFASTSGLQFTIDGETGYFAGTNTYWIGFLTDNADVDLVMGHLKSSGLKILRVWGFNDVTSQPSSGTVWYQLHQDGKSTINTGADGLQRLDYVVSSAEQHDIKLIINFVNYWTDYGGMSAYVSAYGGSGETDFYTSDTMQSAYQTYIKTVVERYSNSSAVFAWELANEPRCPSCDTSVLYNWIEKTSKFIKGLDADRMVCIGDEGFGLNIDSDGSYPYQFSEGLNFTMNLGIDTIDFGTLHLYPDSWGTSDDWGNGWITAHGAACKAAGKPCLLEEYGVTSNHCSVEGSWQKTALSTTGVGADLFWQYGDDLSTGKSPDDGNTIYYGTSDYQCLVTDHVAAIGSA

SEQ ID NO: 4 - protein, 345 aa, synthetic construct
  REGION 1..345: note = Mannanase variant
SFASTSGLQFTIDGETGYFAGTNSYWIGFLTDNADVDLVMGHLKSSGLKILRVWGFNDVTSQPSSGTVWYQLHQDGKSTINTGADGLQRLDYVVSSAEQHDIKLIINFVNYWTDYGGMSAYVSAYGGSGVTDFYTSDTMQSAYQTYIKTVVERYSNSSAVFAWELANEPRCPSCDTSVLYNWIEKTSKFIKGLDADRMVCIGDEGFGLNIDSDGSYPYQFSEGLNFTMNLGIDTIDFGTLHLYPDSWGTSDDWGNGWITAHGAACKAAGKPCLLEEYGVTSNHCSVEGSWQKTALSTTGVGADLFWQYGDDLSTGKSPDDGNTIYYGTSDYQCLVTDHVAAIGSA

SEQ ID NO: 5 - protein, 345 aa, synthetic construct
  REGION 1..345: note = Mannanase variant
SFASTSGLQFTIDGETGYFAGTNSYWIGFLTDNADVDLVMGHLKSSGLKILRVWGFNDVTSQPSSGTVWYQLHQDGKSTINTGADGLQRLDYVVSSAEQHDIKLIINFVNYWTDYGGMSAYVSAYGGSGETDFYTSDTMQSAYQTYIKTVVERYSNSSAVFAWELANEPRCPSCDTSVLYNWIEKTSKFIKGLDADRMVCIGDEGFGLNIDSDGSYPYQFSEGLNFTMNLGIDTIDFGTLHLYPDSWGTSDDWGNGWITAHCAACKAAGKPCLLEEYGVTSNHCSVEGSWQKTALSTTGVGADLFWQYGDDLSTGKSPDDGNTIYYGTSDYQCLVTDHVAAIGSA

SEQ ID NO: 6 - protein, 345 aa, synthetic construct
  REGION 1..345: note = Mannanase variant
SFASTSGLQFTIDGETGYFAGTNTYWIGFLTDNADVDLVMGHLKSSGLKILRVWGFNDVTSQPSSGTVWYQLHQDGKSTINTGADGLQRLDYVVSSAEQHDIKLIINFVNYWTDYGGMSAYVSAYGGSGVTDFYTSDTMQSAYQTYIKTVVERYSNSSAVFAWELANEPRCPSCDTSVLYNWIEKTSKFIKGLDADRMVCIGDEGFGLNIDSDGSYPYQFSEGLNFTMNLGIDTIDFGTLHLYPDSWGTSDDWGNGWITAHGAACKAAGKPCLLEEYGVTSNHCSVEGSWQKTALSTTGVGADLFWQYGDDLSTGKSPDDGNTIYYGTSDYQCLVTDHVAAIGSA

SEQ ID NO: 7 - protein, 383 aa, synthetic construct
  REGION 1..383: note = Mannanase
MKLSNALLTLASLALANVSTALPKASPAPSTSSSAASTSFASTSGLQFTIDGETGYFAGTNSYWIGFLTDNADVDLVMGHLKSSGLKILRVWGFNDVTSQPSSGTVWYQLHQDGKSTINTGADGLQRLDYVVSSAEQHDIKLIINFVNYWTDYGGMSAYVSAYGGSGETDFYTSDTMQSAYQTYIKTVVERYSNSSAVFAWELANEPRCPSCDTSVLYNWIEKTSKFIKGLDADRMVCIGDEGFGLNIDSDGSYPYQFSEGLNFTMNLGIDTIDFGTLHLYPDSWGTSDDWGNGWITAHGAACKAAGKPCLLEEYGVTSNHCSVEGSWQKTALSTTGVGADLFWQYGDDLSTGKSPDDGNTIYYGTSDYQCLVTDHVAAIGSA

SEQ ID NO: 8 - DNA, 1149 bp, synthetic construct
  misc_feature 1..1149: note = Mannanase
  source 1..1149: mol_type = other DNA
atgaagctttccaacgccctcctcaccctggctagcctggcgctggccaacgtctccacggctctgccgaaagcctcccctgcaccgagcaccagcagcagtgctgcctccaccagcttcgccagcacttctgggcttcaatttaccatcgacggtgagacaggctacttcgcgggtacaaattcttactggatcggattcttgaccgataatgccgacgttgaccttgtgatgggtcatcttaagagtagtgggttaaaaattcttagagtctgggggttcaatgatgtgacttcgcagccctccagcggaaccgtgtggtaccaacttcatcaggatggaaagtccactattaacacgggcgcggatggcttgcagcgcctggactacgttgtatcgagcgccgagcaacacgatatcaaacttatcataaacttcgtaaattattggacagattacggtggaatgtcagcgtacgttagcgcttacggtggatctggtgaaacagacttttacacttcagacacgatgcagtcagcctatcagacctatattaagaccgtagtggaacgctactcgaattcatcagcggtgtttgcgtgggaattggcaaatgagccacgttgcccctcttgcgatactagtgttctttacaactggattgaaaagacatcaaaattcatcaaaggtctggacgcagacagaatggtttgtatcggagatgagggcttcggattaaacatcgactctgacgggtcatatccatatcaattctccgaagggttaaattttactatgaacttagggatagacactattgatttcggtacgctgcacttgtaccctgactcctggggcacctcggatgattggggaaatggctggataacggctcatggtgcggcatgcaaggccgctggaaaaccatgtttattagaggagtacggcgtcacaagcaatcattgcagcgtggaaggtagttggcaaaagacagcactgtcaaccacaggggtcggcgcggacctgttttggcagtacggggatgacttaagcacaggaaagtcccccgatgatggaaatacaatatactacggtacatctgattaccagtgcctggttactgaccatgtcgccgccatcggctctgca

SEQ ID NO: 9 - DNA, 37 bp, synthetic construct
  misc_feature 1..37: note = ORF(AnMAN)-F
  source 1..37: mol_type = other DNA
ttcgtgatatactgataataaattgaattttcacact

SEQ ID NO: 10 - DNA, 22 bp, synthetic construct
  misc_feature 1..22: note = ORF(AnMAN)-R
  source 1..22: mol_type = other DNA
aaacagccaagcttgcatgcct

SEQ ID NO: 11 - DNA, 21 bp, synthetic construct
  misc_feature 1..21: note = Vector-F
  source 1..21: mol_type = other DNA
atgcaagcttggctgttttgg

SEQ ID NO: 12 - DNA, 29 bp, synthetic construct
  misc_feature 1..29: note = Vector-R
  source 1..29: mol_type = other DNA
attatcagtatatcacgaacaaaaaagag

SEQ ID NO: 13 - DNA, 27 bp, synthetic construct
  misc_feature 1..27: note = SEQ ID NO: 3-N
  source 1..27: mol_type = other DNA
gcgggtacaaatacctactggatcgga

SEQ ID NO: 14 - DNA, 27 bp, synthetic construct
  misc_feature 1..27: note = SEQ ID NO: 3-R
  source 1..27: mol_type = other DNA
tccgatccagtaggtatttgtacccgc

SEQ ID NO: 15 - DNA, 27 bp, synthetic construct
  misc_feature 1..27: note = SEQ ID NO: 4-N
  source 1..27: mol_type = other DNA
ggtggatctggtgtgacagacttttac

SEQ ID NO: 16 - DNA, 27 bp, synthetic construct
  misc_feature 1..27: note = SEQ ID NO: 4-R
  source 1..27: mol_type = other DNA
gtaaaagtctgtcacaccagatccacc